European Patent Application EP 4 650 362 A1, published November 19, 2025. Title: NEUROPROTECTIVE PSD-95 POLYPEPTIDE INHIBITOR AND USE THEREOF. Applicant: BEIJING TUO JIE BIOPHARMACEUTICAL CO., LTD. Application WO, filed January 9, 2024. The sequence listing filed with the application follows.

SEQUENCE LISTING (67 sequences)

SEQ ID NO: 1 - protein, 9 aa, synthetic construct
  SITE 2: note = X is Aib
  SITE 3: note = X is Dab
  SITE 5..6: note = XX is Tle-Tle
GXXTXXTDV

SEQ ID NO: 2 - skipped

SEQ ID NO: 3 - protein, 8 aa, synthetic construct
  SITE 1: note = X is Nle
  SITE 4..5: note = XX is Tle-Tle
XTTXXTDV

SEQ ID NO: 4 - protein, 7 aa, synthetic construct
  SITE 2..3: note = XX is homoArg-homoArg
TXXITDV

SEQ ID NO: 5 - protein, 9 aa, synthetic construct
  SITE 2: note = X is Aib
  SITE 3..6: note = XXXX is Dab-homoArg-Tle-Tle
GXXXXXTDV

SEQ ID NO: 6 - protein, 9 aa, synthetic construct
  SITE 2: note = X is Aib
  SITE 3: note = X is Dab
  SITE 5..6: note = XX is Chg-Tle
GXXTXXSDV

SEQ ID NO: 7 - protein, 7 aa, synthetic construct
  SITE 3..4: note = XX is Tle-Tle
GTXXTDV

SEQ ID NO: 8 - protein, 7 aa, synthetic construct
  SITE 3..4: note = XX is Chg-Tle
GTXXSDV

SEQ ID NO: 9 - protein, 9 aa, synthetic construct
  SITE 1..9: note = An amino acid residue is optionally a D-amino acid
RKKRRQRRR

SEQ ID NO: 10 - protein, 10 aa, synthetic construct
  SITE 1..10: note = An amino acid residue is optionally a D-amino acid
GRKKRRQRRR

SEQ ID NO: 11 - protein, 11 aa, synthetic construct
  SITE 1..11: note = An amino acid residue is optionally a D-amino acid
YGRKKRRQRRR

SEQ ID NO: 12 - protein, 11 aa, synthetic construct
  SITE 1: note = D-amino acid
  SITE 3..11: note = D-amino acids
YGRKKRRQRRR

SEQ ID NO: 13 - protein, 9 aa, synthetic construct
  SITE 1: note = D-amino acid
  SITE 5: note = D-amino acid
  SITE 9: note = D-amino acid
RKKRRQRRR

SEQ ID NO: 14 - protein, 20 aa, synthetic construct
  SITE 1: note = D-amino acid
  SITE 3..11: note = D-amino acids
  SITE 13: note = X is Aib
  SITE 14: note = X is Dab
  SITE 16..17: note = XX is Tle-Tle
YGRKKRRQRRRGXXTXXTDV

SEQ ID NO: 15 - protein, 17 aa, synthetic construct
  SITE 1: note = D-amino acid
  SITE 3..11: note = D-amino acids
  SITE 12: note = X is AAEA
  SITE 13..14: note = XX is Tle-Tle
YGRKKRRQRRRXXXTDV

SEQ ID NO: 16 - protein, 19 aa, synthetic construct
  SITE 1: note = D-amino acid
  SITE 3..11: note = D-amino acids
  SITE 12: note = X is Nle
  SITE 15..16: note = XX is Tle-Tle
YGRKKRRQRRRXTTXXTDV

SEQ ID NO: 17 - protein, 18 aa, synthetic construct
  SITE 1: note = D-amino acid
  SITE 3..11: note = D-amino acids
  SITE 13..14: note = XX is homoArg-homoArg
YGRKKRRQRRRTXXITDV

SEQ ID NO: 18 - protein, 20 aa, synthetic construct
  SITE 1: note = D-amino acid
  SITE 3..11: note = D-amino acids
  SITE 13: note = X is Aib
  SITE 14..17: note = XXXX is Dab-homoArg-Tle-Tle
YGRKKRRQRRRGXXXXXTDV

SEQ ID NO: 19 - protein, 20 aa, synthetic construct
  SITE 1: note = D-amino acid
  SITE 3..11: note = D-amino acids
  SITE 13: note = X is Aib
  SITE 14: note = X is Dab
  SITE 16..17: note = XX is Chg-Tle
YGRKKRRQRRRGXXTXXSDV

SEQ ID NO: 20 - protein, 18 aa, synthetic construct
  SITE 1: note = D-amino acid
  SITE 3..11: note = D-amino acids
  SITE 14..15: note = XX is Tle-Tle
YGRKKRRQRRRGTXXTDV

SEQ ID NO: 21 - protein, 18 aa, synthetic construct
  SITE 1: note = D-amino acid
  SITE 3..11: note = D-amino acids
  SITE 14..15: note = XX is Chg-Tle
YGRKKRRQRRRGTXXSDV

SEQ ID NO: 22 - protein, 18 aa, synthetic construct
  SITE 1: note = D-amino acid
  SITE 5: note = D-amino acid
  SITE 9: note = D-amino acid
  SITE 11: note = X is Aib
  SITE 12: note = X is Dab
  SITE 14..15: note = XX is Tle-Tle
RKKRRQRRRGXXTXXTDV

SEQ ID NO: 23 - protein, 7 aa, synthetic construct
  SITE 3: note = X is Tle
SSXISTV

SEQ ID NO: 24 - protein, 5 aa, synthetic construct
  SITE 1: note = X is Tle
XISTV

SEQ ID NO: 25 - skipped

SEQ ID NO: 26 - protein, 7 aa, synthetic construct
GSTESWV

SEQ ID NO: 27 - protein, 7 aa, synthetic construct
  SITE 3: note = X is Orn
GSXESWV

SEQ ID NO: 28 - protein, 7 aa, synthetic construct
  SITE 2..3: note = D-amino acids
SRRISTV

SEQ ID NO: 29 - protein, 7 aa, synthetic construct
  SITE 2..3: note = XX is homoArg-homoArg
SXXISTV

SEQ ID NO: 30 - protein, 7 aa, synthetic construct
  SITE 3: note = X is homoArg
GSXESWV

SEQ ID NO: 31 - protein, 7 aa, synthetic construct
  SITE 3: note = X is Orn
  SITE 4: note = X is Tle
GSXXSWV

SEQ ID NO: 32 - protein, 7 aa, synthetic construct
  SITE 3: note = X is Orn
GTXESWV

SEQ ID NO: 33 - protein, 7 aa, synthetic construct
  SITE 3: note = X is Orn
  SITE 6: note = X is Abu
GTXESXV

SEQ ID NO: 34 - protein, 7 aa, synthetic construct
  SITE 3: note = X is Tle
GTXETWV

SEQ ID NO: 35 - protein, 7 aa, synthetic construct
  SITE 2: note = D-amino acid
  SITE 3: note = X is Tle
GKXETWV

SEQ ID NO: 36 - protein, 7 aa, synthetic construct
  SITE 3: note = X is Dab
GTXETWV

SEQ ID NO: 37 - protein, 7 aa, synthetic construct
ARRETAV

SEQ ID NO: 38 - protein, 5 aa, synthetic construct
  SITE 1: note = X is Tle
XETTV

SEQ ID NO: 39 - protein, 9 aa, synthetic construct
  SITE 2: note = X is Aib
  SITE 3: note = X is Dab
  SITE 5: note = X is Tle
GXXTXETTV

SEQ ID NO: 40 - protein, 18 aa, synthetic construct
  SITE 1: note = D-amino acid
  SITE 3..11: note = D-amino acid
  SITE 14: note = X is Tle
YGRKKRRQRRRSSXISTV

SEQ ID NO: 41 - protein, 17 aa, synthetic construct
  SITE 1: note = D-amino acid
  SITE 3..11: note = D-amino acid
  SITE 12: note = X is AEEA
  SITE 13: note = X is Tle
YGRKKRRQRRRXXISTV

SEQ ID NO: 42 - protein, 17 aa, synthetic construct
  SITE 1: note = D-amino acid
  SITE 3..11: note = D-amino acid
  SITE 12: note = X is AEEA
  SITE 13..14: note = XX is Tle-Tle
YGRKKRRQRRRXXXTTV

SEQ ID NO: 43 - protein, 18 aa, synthetic construct
  SITE 1: note = D-amino acid
  SITE 3..11: note = D-amino acid
YGRKKRRQRRRGSTESWV

SEQ ID NO: 44 - protein, 18 aa, synthetic construct
  SITE 1: note = D-amino acid
  SITE 3..11: note = D-amino acid
  SITE 14: note = X is Orn
YGRKKRRQRRRGSXESWV

SEQ ID NO: 45 - protein, 18 aa, synthetic construct
  SITE 1: note = D-amino acid
  SITE 3..11: note = D-amino acid
  SITE 15..16: note = D-amino acid
YGRKKRRQRRRSRRISTV

SEQ ID NO: 46 - protein, 18 aa, synthetic construct
  SITE 1: note = D-amino acid
  SITE 3..11: note = D-amino acid
  SITE 13..14: note = XX is homoArg-homoArg
YGRKKRRQRRRSXXISTV

SEQ ID NO: 47 - protein, 18 aa, synthetic construct
  SITE 1: note = D-amino acid
  SITE 3..11: note = D-amino acid
  SITE 14: note = X is homoArg
YGRKKRRQRRRGSXESWV

SEQ ID NO: 48 - protein, 18 aa, synthetic construct
  SITE 1: note = D-amino acid
  SITE 3..11: note = D-amino acid
  SITE 14: note = X is Orn
  SITE 15: note = X is Tle
YGRKKRRQRRRGSXXSWV

SEQ ID NO: 49 - protein, 18 aa, synthetic construct
  SITE 1: note = D-amino acid
  SITE 3..11: note = D-amino acid
  SITE 14: note = Orn
YGRKKRRQRRRGTXESWV

SEQ ID NO: 50 - protein, 18 aa, synthetic construct
  SITE 1: note = D-amino acid
  SITE 3..11: note = D-amino acid
  SITE 14: note = X is Orn
  SITE 17: note = X is Abu
YGRKKRRQRRRGTXESXV

SEQ ID NO: 51 - protein, 18 aa, synthetic construct
  SITE 1: note = D-amino acid
  SITE 3..11: note = D-amino acid
  SITE 14: note = X is Tle
YGRKKRRQRRRGTXETWV

SEQ ID NO: 52 - protein, 18 aa, synthetic construct
  SITE 1: note = D-amino acid
  SITE 3..11: note = D-amino acid
  SITE 13: note = D-amino acid
  SITE 14: note = X is Tle
YGRKKRRQRRRGKXETWV

SEQ ID NO: 53 - protein, 18 aa, synthetic construct
  SITE 1: note = D-amino acid
  SITE 3..11: note = D-amino acid
  SITE 14: note = X is Dab
YGRKKRRQRRRGTXETWV

SEQ ID NO: 54 - protein, 18 aa, synthetic construct
  SITE 1: note = D-amino acid
  SITE 3..11: note = D-amino acid
YGRKKRRQRRRARRETAV

SEQ ID NO: 55 - protein, 17 aa, synthetic construct
  SITE 1: note = D-amino acid
  SITE 3..11: note = D-amino acid
  SITE 12: note = X is AEEA
  SITE 13: note = X is Tle
YGRKKRRQRRRXXETTV

SEQ ID NO: 56 - protein, 20 aa, synthetic construct
  SITE 1: note = D-amino acid
  SITE 3..11: note = D-amino acid
  SITE 13: note = X is Aib
  SITE 14: note = X is Dab
  SITE 16: note = X is Tle
YGRKKRRQRRRGXXTXETTV

SEQ ID NO: 57 - protein, 18 aa, synthetic construct
  SITE 1..9: note = D-amino acid
  SITE 11: note = X is Aib
  SITE 12: note = X is Dab
  SITE 14..15: note = XX is Tle-Tle
RRRQRRKKRGXXTXXTDV

SEQ ID NO: 58 - protein, 20 aa, synthetic construct
  SITE 1: note = X is Ac-y
  SITE 1: note = D-amino acid
  SITE 3: note = D-amino acid
  SITE 5: note = D-amino acid
  SITE 7: note = D-amino acid
  SITE 9: note = D-amino acid
  SITE 11: note = D-amino acid
  SITE 13..14: note = XX is Aib-Dab
  SITE 16..17: note = XX is Tle-Tle
XGRKKRRQRRRGXXTXXTDV

SEQ ID NO: 59 - protein, 18 aa, synthetic construct
  SITE 1..9: note = D-amino acid
  SITE 11: note = X is Aib
  SITE 12: note = X is Dab
  SITE 14..15: note = XX is Chg-Tle
RRRQRRKKRGXXTXXSDV

SEQ ID NO: 60 - protein, 20 aa, synthetic construct
  SITE 1: note = X is Ac-y
  SITE 1: note = D-amino acid
  SITE 3: note = D-amino acid
  SITE 5: note = D-amino acid
  SITE 7: note = D-amino acid
  SITE 9: note = D-amino acid
  SITE 11: note = D-amino acid
  SITE 13..14: note = XX is Aib-Dab
  SITE 16..17: note = XX is Chg-Tle
XGRKKRRQRRRGXXTXXSDV

SEQ ID NO: 61 - protein, 18 aa, synthetic construct
  SITE 1: note = D-amino acid
  SITE 5: note = D-amino acid
  SITE 9: note = D-amino acid
  SITE 11..12: note = XX is Aib-Dab
  SITE 14..15: note = XX is Chg-Tle
RKKRRQRRRGXXTXXSDV

SEQ ID NO: 62 - protein, 156 aa, synthetic construct
  SITE 1..54: note = Flag-His-Avitag-TEVsite tag, subsequently used for purification and biotinylation
MDYKDDDDKGSHHHHHHHHGGGGSGGGGSGLNDIFEAQKIEWHEGGGGSENLYFQGGGGGSAEKVMEIKLIKGPKGLGFSIAGGVGNQHIPGDNSIYVTKIIEGGAAHKDGRLQIGDKILAVNSVGLEDVMHEDAVAALKNTYDVVYLKVAKPSNA

SEQ ID NO: 63 - protein, 20 aa, synthetic construct
  SITE 1: note = X is Biotin-Y
XGRKKRRQRRRKLSSIESDV

SEQ ID NO: 64 - protein, 20 aa, synthetic construct
  source 1..20: note = NA-1
YGRKKRRQRRRKLSSIESDV

SEQ ID NO: 65 - protein, 20 aa, synthetic construct
  SITE 3: note = D-amino acid
  SITE 7: note = D-amino acid
  SITE 9: note = D-amino acid
  SITE 12: note = D-amino acid
YGRKKRRQRRRKLSSIESDV

SEQ ID NO: 66 - protein, 20 aa, synthetic construct
  source 1..20: note = NA-1(ADA)
YGRKKRRQRRRKLSSIEADA

SEQ ID NO: 67 - protein, 154 aa, synthetic construct
  SITE 1..61: note = Flag-His-Avitag-TEVsite tag, subsequently used for purification and biotinylation
MDYKDDDDKGSHHHHHHHHGGGGSGGGGSGLNDIFEAQKIEWHEGGGGSENLYFQGGGGGSREPRRIVIHRGSTGLGFNIVGGEDGEGIFISFILAGGPADLSGELRKGDQILSVNGVDLRNASHEQAAIALKNAGQTVTIIAQYKPEEYSRFE